European Patent Specification EP 2 670 231 B1, published October 23, 2024. Title: ACETYL CO-ENZYME A CARBOXYLASE HERBICIDE RESISTANT PLANTS. Applicant: Colorado Wheat Research Foundation, Inc Ostlie, Michael Haley, Scott Westra, Philip Valdez, Victoria. The sequence listing filed with the application follows.

SEQUENCE LISTING (16 sequences)

SEQ ID NO: 1 - DNA, 1152 bp, Triticum aestivum
cgtgttggatggtctgatgatggcagccctgaacgtgggtttcagtacatttatctgactgaagaagaccatgctcgtattagcacttctgttatagcgcacaagatgcagcttgataatggtgaaattaggtgggttatcgattctgttgtggggaaggaggatgggctaggtgtggagaacatacatggaagtgctgctattgccagtgcctattctagggcctatgaggagacatttacgcttacatttgtgactggacggactgttggaataggagcatatcttgctcgacttggcatacggtgcatacagcgtactgaccagcccattatcctaactgggttctctgccttgaacaagcttcttggccgggaagtttacagctcccacatgcagttgggtggccccaaaattatggcgacaaacggtgttgtccatctgacagtttcagatgaccttgaaggtgtatctaatatattgaggtggctcagctatgttcctgccaacattggtggacctcttcctattacaaaatctttggacccacctgacagacccgttgcttacatccctgagaatacatgcgatcctcgtgctgccatcagtggcattgatgatagccaagggaaatggttggggggcatgttcgacaaagacagttttgtggagacatttgaaggatgggcgaagtcagttgttactggcagagctaaactcggagggattccggtgggtgttatagctgtggagacacagactatgatgcagctcatccctgctgatccaggccagcttgattcccatgagcggtctgttcctcgtgctgggcaagtctggtttccagattcagctactaagacagcgcaggcaatgctggacttcaaccgtgaaggattacctctgttcatccttgctaactggagaggcttctctggtggacaaagagatctttttgaaggaatccttcaggctgggtcaacaattgttgagaaccttaggacatacaatcagcctgcctttgtatatatccccaaggctgcagagctacgtggaggggcttgggtcgtgattgatagcaagataaatccagatcgcattgagttctatgctgagaggactgcaaagggcaatgttctcgaacctcaaggg

SEQ ID NO: 2 - DNA, 1161 bp, Triticum aestivum
atcttgcttccgtgttggatggtctgatgatggcagccctgaacgtgggtttcaatatatttatctgactgaagaagaccatgctcgtattagcgcttctgttatagcgcacaagatgcagcttgataatggtgaaattaggtgggttattgattctgttgtagggaaggaggatgggctaggtgtggagaacatacatggaagtgctgctattgccagtgcctattctagggcctatgaggagacatttacgcttacatttgtgactggaaggactgttggaataggagcatatcttgctcgacttggcatacggtgcattcagcgtactgaccagcccattatcctaactgggttttctgccttgaacaagcttcttggccgggaagtgtacagctcccacatgcagttgggtggccccaaaattatggccacaaacggtgttgtccatctgacagtttcagatgaccttgaaggtgtatctaatatattgaggtggctcagctatgttcctgccaacattggtggacctcttcctattacaaaatctttggacccacctgacagacccgttgcttacatccctgagaatacatgtgatcctcgtgcagccatcagtggcattgatgatagccaagggaaatggttggggggcatgttcgacaaagacagttttgtggagacatttgaaggatgggcgaagtcagtagttactggcagagcgaaactcggagggattccggtgggtgttatagctgtggagacacagactatgatgcagctcatccctgctgatccaggtcagcttgattcccatgagcggtctgttcctcgtgctgggcaagtctggtttccagattcagctactaagacagcgcaggcaatgctggacttcaaccgtgaaggattacctctgttcatccttgctaactggagaggcttctctggtgggcaaagagatctttttgaaggaatccttcaggctgggtcaacaattgttgagaaccttaggacatacaatcagcctgcctttgtatatatccccaaggctgcagagctacgtggaggggcttgggtcgtgattgatagcaagataaatccagatcgcattgagttctatgctgagaggactgcaaagggcaatgttctgaacctcaaggg

SEQ ID NO: 3 - DNA, 1129 bp, Triticum aestivum
gtgttggatggtctgatgatggcagccctgaacgtgggtttcagtacatttatctgactgaagaagaccatgctcgtattagcacttctgttatagcgcacaagatgcagcttgataatggtgaaattaggtgggttattgattctgttgtggggaaggaggatgggctaggtgtggagaacatacatggaagtgctgctattgccagtgcctattctagggcctatgaggagacatttacgcttacatttgtgactggacggactgttggaataggagcatatcttgctcgacttggcatacggtgcatacagcgtactgaccagcccattatcctaaccgggttctctgctttgaacaagcttcttggccgggaagtgtacagctcccacatgcagttgggtggccccaaaattatggcgacaaacggtgttgtccatctgacagtttcagatgaccttgaaggtgtgtctaatatattgaggtggctcagctatgttcctgccaacattggtggacctcttcctattacaaaatctttggacccacctgacagacccgttgcatatatccctgagaatacatgtgatcctcgtgcagccatcagtggcattgatgatagccaagggaaatggttggggggcatgttcgacaaagacagttttgtggagacatttgaaggatgggcgaagtcagtagttactggcagagcgaaactcggagggattccggtgggtgttatagctgtggagacacagactatgatgcagctcatccctgctgatccaggccagcttgattcccatgagcggtctgttcctcgtgctgggcaagtctggtttccagattcagctactaagacagctcaagcaatgctggacttcaaccgtgaaggattacctctgttcatccttgctaactggagaggcttctctggtgggcaaagagatctttttgaaggaatccttcaggctgggtcaacaattgttgagaaccttaggacatacaatcagcctgcctttgtatatatccccaaggctgcagagctacgtggaggggcttgggtcgtgattgatagcaagataaatccagatcgaattgagttctatgctgagaggactgcaaaggg

SEQ ID NO: 4 - DNA, 1188 bp, Triticum aestivum
gatgaagtaaaatcgtgcttcgtgttggatggtctgatgatggcagccctgaacgtgggtttcagtacatttatctgactgaagaagaccatgctcgtattagcacttctgttatagcgcacaagatgcagcttgataatggtgaaattaggtgggttattgattctgttgtggggaaggaggatgggctaggtgtggagaacatacatggaagtgctgctattgccagtgcctattctagggcctatgaggagacatttacgcttacatttgtgactggacggactgttggaataggagcatatcttgctcgacttggcatacggtgcatacagcgtactgaccagcccattatcctaaccgggttctctgctttgaacaagcttcttggccgggaagtgtacagctcccacatgcagttgggtggccccaaaattatggcgacaaacggtgttgtccatctgacagtttcagatgaccttgaaggtgtgtctaatatattgaggtggctcagctatgttcctgccaacattggtggacctcttcctattacaaaatctttggacccacctgacagacccgttgcatatatccctgagaatacatgtgatcctcgtgcagccatcagtggcattgatgatagccaagggaaatggttggggggcatgttcgacaaagacagttttgtggagacatttgaaggatgggcgaagtcagtagttactggcagagcgaaactcggagggattccggtgggtgttatagctgtggagacacagactatgatgcagctcatccctgctgatccaggccagcttgattcccatgagcggtctgttcctcgtgctgggcaagtctggtttccagattcagttactaagacagctcaagcaatgctggacttcaaccgtgaaggattacctctgttcatccttgctaactggagaggcttctctggtgggcaaagagatctttttgaaggaatccttcaggctgggtcaacaattgttgagaaccttaggacatacaatcagcctgcctttgtatatatccccaaggctgcagagctacgtggaggggcttgggtcgtgattgatagcaagataaatccagatcgaattgagttctatgctgagaggactgcaaagggtaatgttcttgaacctcaagggttgattgagataccag

SEQ ID NO: 5 - DNA, 1194 bp, Triticum aestivum
ggcatagcagatgaagtagagtcttgcttccgtgttggatggtctgatgatggcagccctgaacgtgggtttcagtacatttatctgactgaagaagaccatgctcgtattagcacttctgttatagcgcacaagatgcagcttgataatggtgaaattaggtgggttatcgattctgttgtggggaaggaggatgggctaggtgtggagaacatacatggaagtgctgctattgccagtgcctattctagggcctatgaggagacatttacgcttacatttgtgactggacggactgttggaataggagcatatcttgctcgacttggcatacggtgcatacagcgtactgaccagcccattatcctaactgggttctctgccttgaacaagcttcttggccgggaagtttacagctcccacatgcagttgggtggccccaaaattatggcgacaaacggtgttgtccatctgacagtttcagatgaccttgaaggtgtatctaatatattgaggtggctcagctatgttcctgccaacattggtggacctcttcctattacaaaatctttggacccacctgacagacccgttgcttacatccctgagaatacatgcgatcctcgtgctgccatcagtggcattgatgatagccaagggaaatggttggggggcatgttcgacaaagacagttttgtggagacatttgaaggatgggcgaagtcagttgttactggcagagctaaactcggagggattccggtgggtgttatagctgtggagacacagactatgatgcagctcatccctgctgatccaggccagcttgattcccatgagcggtctgttcctcgtgctgggcaagtctggtttccagattcagttactaagacagcgcaggcaatgctggacttcaaccgtgaaggattacctctgttcatccttgctaactggagaggcttctctggtggacaaagagatctttttgaaggaatccttcaggctgggtcaacaattgttgagaaccttaggacatacaatcagcctgcctttgtatatatccccaaggctgcagagctacgtggaggggcttgggtcgtgattgatagcaagataaatccagatcgcattgagttctatgctgagaggactgcaaagggcaatgttctcgaacctcaagggttgattgagatg

SEQ ID NO: 6 - DNA, 1184 bp, Triticum aestivum
tgaagtaaaatcttgcttccgtgttggatggtctgatgatggcagccctgaacgtgggtttcaatatatttatctgactgaagaagaccatgctcgtattagcgcttctgttatagcgcacaagatgcagcttgataatggtgaaattaggtgggttattgattctgttgtagggaaggaggatgggctaggtgtggagaacatacatggaagtgctgctattgccagtgcctattctagggcctatgaggagacatttacgcttacatttgtgactggaaggactgttggaataggagcatatcttgctcgacttggcatacggtgcattcagcgtactgaccagcccattatcctaactgggttttctgccttgaacaagcttcttggccgggaagtgtacagctcccacatgcagttgggtggccccaaaattatggccacaaacggtgttgtccatctgacagtttcagatgaccttgaaggtgtatctaatatattgaggtggctcagctatgttcctgccaacattggtggacctcttcctattacaaaatctttggacccacctgacagacccgttgcttacatccctgagaatacatgtgatcctcgtgcagccatcagtggcattgatgatagccaagggaaatggttggggggcatgttcgacaaagacagttttgtggagacatttgaaggatgggcgaagtcagtagttactggcagagcgaaactcggagggattccggtgggtgttatagctgtggagacacagactatgatgcagctcatccctgctgatccaggtcagcttgattcccatgagcggtctgttcctcgtgctgggcaagtctggtttccagattcagttactaagacagcgcaggcaatgctggacttcaaccgtgaaggattacctctgttcatccttgctaactggagaggcttctctggtgggcaaagagatctttttgaaggaatccttcaggctgggtcaacaattgttgagaaccttaggacatacaatcagcctgcctttgtatatatccccaaggctgcagagctacgtggaggggcttgggtcgtgattgatagcaagataaatccagatcgcattgagttctatgctgagaggactgcaaagggcaatgttcttgaacctcaagggttgattgagatgc

SEQ ID NO: 7 - protein, 375 aa, Triticum aestivum
VGWSDDGSPERGFQYIYLTEEDHARISTSVIAHKMQLDNGEIRWVIDSVVGKEDGLGVENIHGSAAIASAYSRAYEETFTLTFVTGRTVGIGAYLARLGIRCIQRTDQPIILTGFSALNKLLGREVYSSHMQLGGPKIMATNGVVHLTVSDDLEGVSNILRWLSYVPANIGGPLPITKSLDPPDRPVAYIPENTCDPRAAISGIDDSQGKWLGGMFDKDSFVETFEGWAKSVVTGRAKLGGIPVGVIAVETQTMMQLIPADPGQLDSHERSVPRAGQVWFPDSATKTAQAMLDFNREGLPLFILANWRGFSGGQRDLFEGILQAGSTIVENLRTYNQPAFVYIPKAAELRGGAWVVIDSKINPDRIEFYAERTAK

SEQ ID NO: 8 - protein, 394 aa, Triticum aestivum
SKIVLRVGWSDDGSPERGFQYIYLTEEDHARISTSVIAHKMQLDNGEIRWVIDSVVGKEDGLGVENIHGSAAIASAYSRAYEETFTLTFVTGRTVGIGAYLARLGIRCIQRTDQPIILTGFSALNKLLGREVYSSHMQLGGPKIMATNGVVHLTVSDDLEGVSNILRWLSYVPANIGGPLPITKSLDPPDRPVAYIPENTCDPRAAISGIDDSQGKWLGGMFDKDSFVETFEGWAKSVVTGRAKLGGIPVGVIAVETQTMMQLIPADPGQLDSHERSVPRAGQVWFPDSVTKTAQAMLDFNREGLPLFILANWRGFSGGQRDLFEGILQAGSTIVENLRTYNQPAFVYIPKAAELRGGAWVVIDSKINPDRIEFYAERTAKGNVLEPQGLIEIP

SEQ ID NO: 9 - protein, 384 aa, Triticum aestivum
RVGWSDDGSPERGFQYIYLTEEDHARISTSVIAHKMQLDNGEIRWVIDSVVGKEDGLGVENIHGSAAIASAYSRAYEETFTLTFVTGRTVGIGAYLARLGIRCIQRTDQPIILTGFSALNKLLGREVYSSHMQLGGPKIMATNGVVHLTVSDDLEGVSNILRWLSYVPANIGGPLPITKSLDPPDRPVAYIPENTCDPRAAISGIDDSQGKWLGGMFDKDSFVETFEGWAKSVVTGRAKLGGIPVGVIAVETQTMMQLIPADPGQLDSHERSVPRAGQVWFPDSATKTAQAMLDFNREGLPLFILANWRGFSGGQRDLFEGILQAGSTIVENLRTYNQPAFVYIPKAAELRGGAWVVIDSKINPDRIEFYAERTAKGNVLEPQG

SEQ ID NO: 10 - protein, 398 aa, Triticum aestivum
GIADEVESCFRVGWSDDGSPERGFQYIYLTEEDHARISTSVIAHKMQLDNGEIRWVIDSVVGKEDGLGVENIHGSAAIASAYSRAYEETFTLTFVTGRTVGIGAYLARLGIRCIQRTDQPIILTGFSALNKLLGREVYSSHMQLGGPKIMATNGVVHLTVSDDLEGVSNILRWLSYVPANIGGPLPITKSLDPPDRPVAYIPENTCDPRAAISGIDDSQGKWLGGMFDKDSFVETFEGWAKSVVTGRAKLGGIPVGVIAVETQTMMQLIPADPGQLDSHERSVPRAGQVWFPDSVTKTAQAMLDFNREGLPLFILANWRGFSGGQRDLFEGILQAGSTIVENLRTYNQPAFVYIPKAAELRGGAWVVIDSKINPDRIEFYAERTAKGNVLEPQGLIEM

SEQ ID NO: 11 - protein, 386 aa, Triticum aestivum
SCFRVGWSDDGSPERGFQYIYLTEEDHARISASVIAHKMQLDNGEIRWVIDSVVGKEDGLGVENIHGSAAIASAYSRAYEETFTLTFVTGRTVGIGAYLARLGIRCIQRTDQPIILTGFSALNKLLGREVYSSHMQLGGPKIMATNGVVHLTVSDDLEGVSNILRWLSYVPANIGGPLPITKSLDPPDRPVAYIPENTCDPRAAISGIDDSQGKWLGGMFDKDSFVETFEGWAKSVVTGRAKLGGIPVGVIAVETQTMMQLIPADPGQLDSHERSVPRAGQVWFPDSATKTAQAMLDFNREGLPLFILANWRGFSGGQRDLFEGILQAGSTIVENLRTYNQPAFVYIPKAAELRGGAWVVIDSKINPDRIEFYAERTAKGNVLNLK

SEQ ID NO: 12 - protein, 394 aa, Triticum aestivum
EVKSCFRVGWSDDGSPERGFQYIYLTEEDHARISASVIAHKMQLDNGEIRWVIDSVVGKEDGLGVENIHGSAAIASAYSRAYEETFTLTFVTGRTVGIGAYLARLGIRCIQRTDQPIILTGFSALNKLLGREVYSSHMQLGGPKIMATNGVVHLTVSDDLEGVSNILRWLSYVPANIGGPLPITKSLDPPDRPVAYIPENTCDPRAAISGIDDSQGKWLGGMFDKDSFVETFEGWAKSVVTGRAKLGGIPVGVIAVETQTMMQLIPADPGQLDSHERSVPRAGQVWFPDSVTKTAQAMLDFNREGLPLFILANWRGFSGGQRDLFEGILQAGSTIVENLRTYNQPAFVYIPKAAELRGGAWVVIDSKINPDRIEFYAERTAKGNVLEPQGLIEM

SEQ ID NO: 13 - DNA, 12753 bp, Alopecurus myosuroides Huds
tcagtttatggcagtctgtgtttgaagaacactgcaactccgctgtctgtccaaagggaggacgatgggatccacacatctgcccattgtcgggtttaatgcatccacaacaccatcgctatccactcttcgccagataaactcagctgctgctgcattccaatcttcgtccccttcaaggtcatccaagaagaaaagccgacgtgttaagtcaataagggatgatggcgatggaagcgtgccagaccctgcaggccatggccagtctattcgccaaggtgaacccaggaccatctccttacttttttgtcgtcaacctcagacttgcatagatttactttcttgattgagagcatgcttgttttagtgtaagatatctcaatactgtatcacaaaatgatagttaagaacaaaccactacaccaatcttcacatattgttcttattgggtttgctaaatcttagttcgcattagatttttttatgtctatgtcgacaccctgagcctccccgtgtctctgcattgagattcaagcagggataggggaaatcacgactggatccttagccataattaaatctctgtcaacttaggtgtagatggactctgtttttaatattcagtatgatgttttcttaagggagagggacacaaaaatacatgtatgttgcagtttaagaatttatgactgaatgttttgatgatataatagttctggaaaagaaggatgcctagattttgtatttttgataaatgtagttataaaattcgaaaggttggcaaaccattgcttcttcttagctattgtgttggcttgctcagtttccaatgcatatctggatgtaggtctcgctggcatcatcgacctcccaaaggagggcgcatcagctccagatgtggacatttcacagtaagtacctcagcacactcacattatagcttagtcctcttgaaagaacaggcaaaaatgtataacgcatgtataattcctagatttcacttgtcttattatcgttacgctgaaatgttgaagttgtaaattcgttattctcatagatttacacctctatgtacatcatagttatgcactatgcacctgctgtgagttctggaaattgaaccattcagcgcactgcaatctgtaaggttttgtttttatataatatggttataaatcatgttcaacctctgcatctacaacattatttatgtgtggtatagtatatagtaatgttacagggtgagattttgctatataagttatgaaacttgtgtttaactttgtaaagggaaacatcctcaaacctgttcttagtggttacagcccaggcacatggccgttgcactgtatggagtattgttgggcacttacagaacattttattggaaagactttttcatataagtattgtttaaatttaattgccaactgaaacccttacccggataacaagatgaataacccacttgcgtttttgattcatactaggcattactatgtcatatgtattacggtgaccgcagtaataactttgctctttcttttctagtgggtctgaagaccacaaggcctcctaccaaatgaatgggatactgaatgaatcacataacgggaggcacgcctctctgtctaaagtttatgaattttgcacggaattgggtggaaaaacaccaattcacagtgtattagtcgccaacaatggaatggcagcagctaagttcatgcggagtgtccggacatgggctaatgatacatttgggtcagagaaggcgattcagttgatagctatggcaactccggaagacatgagaataaatgcagagcacattagaattgctgatcagtttgttgaagtacctggtggaacaaacaataacaactatgcaaatgtccaactcatagtggaggtcagtactggtcatcccttgatgtgcagttatgcacaagctcctctttggtctttagcatgacatggcaacttcacttttgcagatagcagagagaactggtgtctccgccgtttggcctggttggggccatgcatctgagaatcctgaacttccagatgcactaactgcaaaaggaattgtttttcttgggccaccagcatcatcaatgaacgcactaggcgacaaggttggttcagctctcattgctcaagcagcaggggttcccactcttgcttggagtggatcacatgtaagcctcacattctctctgataaatcatcacctgatatttatggtggatgcattatgtaacctatgacatttttattctaggtggaaattccattagaactttgtttggactcgatacctgaggagatgtataggaaagcctgtgttacaaccgctgatgaagcagttgcaagttgtcagatgattggttaccctgccatgatcaaggcatcctggggtggtggtggtaaagggattagaaaggtacattattcatttgattggactgtacacaagagattgtgtgggctgtgatattttgtgcacagtgttagccctaacctttttaacatattaactcgatatctcttgcaggttaataatgatgacgaggtgaaagcactgtttaagcaagtacagggtgaagttcctggctccccgatatttatcatgagacttgcatctcaggttagacttctctggaagttctattttccaagcgtgctgtatctgggttgtatattgtacgtatggaagctttatttgctctttcttacaggctaaaattgtatcctgtaatctgtactaatattgtaattttcatttaaatccctctcccctttccttttgtagagtcgtcatcttgaagtccagctgctttgtgatgaatatggcaatgtagcagcacttcacagtcgtgattgcagtgtgcaacgacgacaccaaaaggtatgctgctccaaactgaaatcatcacttttatttcggttctgctttacgtgtagttttgatcaaatggttcaactgtgtccattttgtttgtttataacagattatcgaggaaggaccagttactgttgctcctcgtgaaacagtgaaagagctagagcaagcagcaaggaggcttgctaaggccgtgggttacgtcggtgctgctactgttgaatatctctacagcatggagactggtgaatactattttctggagcttaatccacggttgcaggtttgttcttttggacactctccaggacttctattttgttggcagtcgtttacattgttaaatggtctatattcaggttgagcacccagtcaccgagtcgatagctgaagtaaatttgcctgcagcccaagttgcagttgggatgggtatacccctttggcagattccaggtaataataatatcattgtaaagagtttcgtttctgtcccatgttctttctgtctaactatctccttattcagagatcagacgtttctacggaatggacaatggaggaggctatgatatttggaggaaaacagcagctctcgctactccattcaactttgatgaagtagattctcaatggccgaagggtcattgtgtggcagttaggataaccagtgagaatccagatgatggattcaagcctactggtggaaaagtaaaggtgggatttcctaatgttatatctatgtttcaattacactacggttagtaaactgatctgatcttgatttttttcgtatatttcaggagataagttttaaaagtaagccaaatgtctggggatatttctcagttaaggtaagctgttcatagctctgttgcagggtcatcttgttttgagttccgcagaagattagtctgcaagatttttattcgaattagtattctcattttggtttttgactaagtattgatccaatcaacaaatattgtctctcccttcatctgttttcagtctggtggaggcattcatgaatttgcggattctcagtttggtatgtaaaatgtaacgtaatgaatattcctctttgctattcgtactgatccttacattggaattgctcctttcattacaggacacgtttttgcctatggagagactagatcagcagcaataaccagcatgtctcttgcactaaaagagattcaaattcgtggagaaattcatacaaacgttgattacacggttgatctcttgaatgtaagtaacaataacaatttgttgaatcctacttttgatgtgatacaaccattttacatccggctttccttcaaaataatcccattctgtggtttctcgtatctttaattcaggccccagacttcagagaaaacacgatccataccggttggctggataccagaatagctatgcgtgttcaagctgagaggcctccctggtatatttcagtggttggaggagctctatatgtaagatatgaaactatgttaatgttactgcaacttttggcaagccaatcttgaaaaacactagtgtttaattgaaataattgttttgtgctgtagaaaacaataaccaccaatgcggagaccgtttctgaatatgttagctatctcatcaagggtcagattccaccaaaggtagtgtcttaatgggcttaaactctgtatattgcttgaaggtggacattgctgaccagtgtttttgtgcagcacatatcccttgtccattcaactatttctttgaatatagaggaaagcaaatatacagtaagtgtgacattccttaaaaaaagactctcagttacaatgaaatgatacttacactgatgctcatctacaccatgccacagattgagattgtgaggagtggacagggtagctacagattgagactgaatggatcacttattgaagccaatgtacaaacattatgtgatggaggccttttaatgcaggtaccttctttcttttacttgctcataaatgtgatataatgtctgctgaaatagttctgattctttagttgtaatgtctccagctggatggaaatagccatgttatttatgctgaagaagaagcgggtggtacacggcttcttattgatggaaaaacatgcttgctacaggtaagaatattctgtttgtttgctcctttataatcttagtgtttgatggtaggactttatattcttatttgtgactttttagagcatccacaacccaaagcgcttaggtagacgcttaaatacaaaaaaataaatacttaaaaagagtaaaacggataagagttgctacctgcaacgcccggcgcttaatctgaggcgcttaatccggtatagctacaggccgtcgctgcctttttgctgcaaaaagaaagggtaagcgtcaggcgcatactttggcgtcgatgtcatcccgacgctaggatttgtgggcataaccgtcgggttggccaggattttcttcctagcatcggaggctaagcgccccgttgtggctgctcttactgcattcacctcttgaccattagcacttcattttttacacttcatctgtattgcttctgctgtttctcaattatagttattccaatgaccactctttagtaattttaacaattgccaatttatcataatacggggcaaaaaagtaggcgtccttaacaccatgtcatgtaacctataataagcttgtgataaaatcatttgtgatacaatagaacagttgaatactttatgatttctttcttacatgaatactttatgattcttgatgacgctgcactgtatcctaagctacataaattacaaatcgttttgcagaatgaccatgatccgtcaaggttattagctgagacaccctgcaaacttcttcgtttcttgattgccgatggtgctcatgttgatgctgatgtaccatacgcggaagttgaggttatgaagatgtgcatgcccctcttgtcgcctgctgctggtgtcattaatgttttgttgtctgagggccaggcgatgcaggttatattactgcccttttgttgcttctgctgttaaaagccattgcatgcgaagcatctgaacttaatatattttgtttcaggctggtgatcttatagcgagacttgatctcgatgacccttctgctgtgaagagagccgagccatttgaaggatcttttccagaaatgagccttcctattgctgcttctggccaagttcacaaaagatgtgctgcaagtttgaacgctgctcgaatggtccttgcaggatatgaccatgcggccaacaaagtaaacatcaagacattttatctcatgtttcctgcttttctcaaataccattctttaatagtatgaattctggattattctgacttattggcattttctgccttttgctaccaaatggtttctaatctatagaagttcttgagcttgtctttgcaaatcttgatttaatgcttttcttgtatgttcatcatactcatttatgataggttgcatttatccttctgctattttcctttctctcagtaaatcatgatggatgctctttctgttatgttcatcatgctgtctattatccttgtgctatttttctatttccagtagtggatgtattggtttaataattcctgatcaaactttgtattttgttgttatttatacttggctcccttttcaggttgtgcaagatttggtatggtgccttgatacacctgctcttcctttcctacaatgggaagagcttatgtctgttttagcaactagacttccaagacgtcttaagagcgaggtatgtgataattgatatgatatgcagaatcaggcataaagggacattgatacatttaatttatgatatagaagggtcttcatcctcgattaaaagatcaattcacttatcatgatttacattctacattgttgaatcaccttggtaatttgccgtaacttattgggcaactattagcttttctaataacgtaatcaaaattcagaatattttacttcaattcttcgtaacatggaacatttggtacttcgtctcatttatttgcactgtacgctgttttagttggtttgccattctaactgaatctttaaagttcttacttatttggttttaacccagatcttgtttatttatcttttataactttcttatgttctgcctcaacggtttatactttttatgcatccagttggagggcaaatacaatgaatacaagttaaatgttgaccatgtgaagatcaaggatttccctaccgagatgcttagagagacaatcgaggtcagtttttgtttcttatggcaccccagtctaaattatactattttttgtaacaagttttcttttaggaaaatcttgcatgtgtttccgagaaggaaatggtgacaattgagaggcttgttgaccctctgatgagcctgctgaagtcatacgagggtgggagagaaagccatgcccactttattgtcaagtccctttttgaggagtatctctcggttgaggaactattcagtgatggcattcaggttatctaacacttctaaactgagcagatctactagagtcattttctaagggtcataattttccagaacctcttgggtgattaagtagcaaaaataatttgtacacgacttacgacttgcttccttcgaaacacttttcactcattattttcctcaaaatgtgccattttgtagtctgacgtgattgaacgcctgcgcctacaatatagtaaagacctccagaaggttgtagacattgttttgtctcaccaggtaaactactttttggcctaatgacttggtgcaaatgatcacagaaacaatctttgttactgatagtttgatttgttctagggtgtgagaaacaaaacaaagctgatactcgcgctcatggagaaactggtctatccaaaccctgctgcctacagagatcagttgattcgcttttcttccctcaaccataaaagatattataaggtgacaatggcgacctaaagtaatggaagctttttgattaatttgttgtgatattttaggctaatgaattactttcattgtaattatgcagttggctcttaaagctagtgaacttcttgaacaaaccaagctcagcgaactccgcacaagcattgcaaggaacctttcagcgctggatatgttcaccgaggaaaaggcagatttctccttgcaagacagaaaattggccattaatgagagcatgggagatttagtcactgccccactgccagttgaagatgcacttgtttctttgtttgattgtactgatcaaactcttcagcagagagtgattgagacatacatatctcgattataccaggtattacatgagctatttttttctggattttattatactctctctcagcatttctggaagcataaactaaggttcctaatgaaataagatactcagtgtttcattaagataaatcctagataatctaggcgtgggaagatttgatttagaacttgtaggcatgttactgctctgtaagttggctaacttgccaatgatattttcagcctcaacttgtgaaggatagcatccagctgaaatatcaggattctggtgttattgctttatgggaattcactgaaggaaatcatgagaagagattgggtgctatggttatcctgaagtcactagaatctgtgtcaacagccattggagctgctctaaaggatgcatcacattatgcaagctctgcgggcaacacggtgcatattgctttgttggatgctgatacccaactgaatacaactgaagataggtatgttcatgtgcagtattagtgcagatgagtttatttggtgcaaaaataagttaatctatttctttcagtggtgataatgaccaagctcaagacaagatggataaactttcttttgtactgaaacaagatgttgtcatggctgatctacgtgctgctgatgtcaaggttgttagttgcattgttcaaagagatggagcaatcatgcctatgcgccgtaccttcctcttgtcagaggaaaaactttgttacgaggaagagccgattcttcggcatgtggagcctccactttctgcacttcttgagttggtatgcaactccatcaaactgactacgtgctgttttgatatattttaatgctttcattttgttatttgctacttgtattcacttagcttgctgtggatacaggataaattgaaagtgaaaggatacaatgagatgaagtatacaccgtcacgtgatcgtcagtggcatatatacacacttagaaatactgaaaatccaaaaatgctgcacagggtatttttccgaacacttgtcagacaacccagtgcaggcaacaggtttacatcagaccatatcactgatgttgaagtaggacatgcagaggaacctctttcatttacttcaagcagcatattaaaatcgttgatgattgctaaagaagaattggagcttcacgcgatcaggactggccattctcatatgtacttgtgcatattgaaagagcaaaagcttcttgaccttgttcctgtttcagggtaagcctgcacatcgttctttttgcagaacatgtattccttgctcttgtgttctgccttctcaatgagcttttcatcgtactcaggaacactgttgtggatgttggtcaagatgaagctactgcatgctctcttttgaaagaaatggctttaaagatacatgaacttgttggtgcaagaatgcatcatctttctgtatgccagtgggaagtgaaacttaagttggtgagcgatgggcctgccagtggtagctggagagttgtaacaaccaatgttactggtcacacctgcactgtggatgtgagttttatctccttgcttcctgtttttctgcatggaactaatgaaactgaagtgaacatattatatatgtgacatacataggactatcatctttgattatcataaaaaaagaactatcatcttcgtttcgtttgttgtcatttccacctcatttttggtctgaatctcatggtgcttttaatgcttttagatctaccgggaggtcgaagatacagaatcacagaaactagtataccactccaccgcattgtcatctggtcctttgcatggtgttgcactgaatacttcgtatcaacctttgagtgttattgatttaaaacgttgctctgccaggaacaacaaaactacatactgctatgattttccattggttagtatctatctctatatgtattatgttagcaggttcttattggtattacatgtcctaaatctgacaacaactcaaaatgtagacatttgaagctgcagtgcagaagtcgtggtctaacatttccagtgaaaacaaccaatgttatgttaaagcgacagagcttgtgtttgctgaaaagaatgggtcgtggggcactcctataattcctatgcagcgtgctgctgggctgaatgacattggtatggtagcctggatcttggacatgtccactcctgaatttcccagcggcagacagatcattgttatcgcaaatgatattacatttagagctggatcatttggcccaagggaagatgcatttttcgaagctgtaaccaacctggcttgtgagaagaagcttccacttatctacttggctgcaaactctggtgctcggattggcattgctgatgaagtaaaatcttgcttccgtgttggatggactgatgatagcagccctgaacgtggatttaggtacatttatatgactgacgaagaccatgatcgtattggctcttcagttatagcacacaagatgcagctagatagtggcgagatcaggtgggttatcgattctgttgtgggaaaagaggatggactaggtgtggagaacatacatggaagtgctgctattgccagtgcctattctagggcgtacgaggagacatttacacttacattcgttactggacgaactgttggaatcggagcctatcttgctcgacttggcatacggtgcatacagcgtattgaccagcccattattttgactgggttttctgccctgaacaagcttcttgggcgggaggtgtacagctcccacatgcagttgggtggtcccaaaatcatggcgacgaatggtgttgtccatctgactgttccagatgaccttgaaggtgtttctaatatattgaggtggctcagctatgttcctgcaaacattggtggacctcttcctattacaaaatctttggacccaatagacagacccgttgcatacatccctgagaatacatgtgatcctcgtgcagccatcagtggcattgatgacagccaagggaaatggttgggtggcatgtttgacaaagacagttttgtggagacatttgaaggatgggcgaagacagtagttactggcagagcaaaacttggagggattcctgttggtgttatagctgtggagacacagaccatgatgcagctcgtccccgctgatccaggccagcctgattcccacgagcggtctgttcctcgtgctgggcaagtttggtttccagattctgctaccaagacagcgcaggcgatgttggacttcaaccgtgaaggattacctctgttcatacttgctaactggagaggcttctctggagggcaaagagatctttttgaaggaaatctgcaggctgggtcaacaattgttgagaaccttaggacatacaatcagcctgcctttgtatatatccccaaggctgcagagctacgtggaggagcctgggtcgtgattgatagcaagataaacccagatcgcatcgagtgctatgctgagaggactgcaaagggtaatgttctcgaacctcaagggttgattgagatcaagttcaggtcagaggaactcaaagaatgcatgggtaggcttgatccagaattgatagatctgaaagcaagactccagggagcaaatggaagcctatctgatggagaatcccttcagaagagcatagaagctcggaagaaacagttgctgcctctgtacacccaaatcgcggtacgttttgcggaattgcacgacacttcccttagaatggctgctaaaggtgtgatcaggaaagttgtagactgggaagactctcggtctttcttctacaagagattacggaggaggctatccgaggacgttctggcaaaggagattagaggtgtaattggtgagaagtttcctcacaaatcagcgatcgagctgatcaagaaatggtacttggcttctgaggcagctgcagcaggaagcaccgactgggatgatgacgatgcttttgtcgcctggagggagaaccctgaaaactataaggaatatatcaaagagcttagggctcaaagggtatctcggttgctctcagatgttgcaggctccagttcggatttacaagccttgccgcagggtctttccatgctactagataaggtacgcatacttacagttttacctgcatctgtttatttgcaagtattttatcgaggttgagtatgtcctgctatcttattcaaatatagtatcttaccaaataatatctaagacgctggatactttgttcagatggatccctctaagagagcacagtttatcgaggaggtcatgaaggtcctgaaatgatcaaatgataccaacacatccaatacagtatgtgcatgatatctgtttctcttgaagtacatatatagatggatacaaggcggctgtaactgatggtagctaatctgggccaaccattacttttgtgaacttgctggtggtctttattattcaaggcacagctcgccttcggaccccctc

SEQ ID NO: 14 - protein, 2320 aa, Alopecurus myosuroides Huds
MGSTHLPIVGFNASTTPSLSTLRQINSAAAAFQSSSPSRSSKKKSRRVKSIRDDGDGSVPDPAGHGQSIRQGLAGIIDLPKEGASAPDVDISHGSEDHKASYQMNGILNESHNGRHASLSKVYEFCTELGGKTPIHSVLVANNGMAAAKFMRSVRTWANDTFGSEKAIQLIAMATPEDMRINAEHIRIADQFVEVPGGTNNNNYANVQLIVEIAERTGVSAVWPGWGHASENPELPDALTAKGIVFLGPPASSMNALGDKVGSALIAQAAGVPTLAWSGSHVEIPLELCLDSIPEEMYRKACVTTADEAVASCQMIGYPAMIKASWGGGGKGIRKVNNDDEVKALFKQVQGEVPGSPIFIMRLASQSRHLEVQLLCDEYGNVAALHSRDCSVQRRHQKIIEEGPVTVAPRETVKELEQAARRLAKAVGYVGAATVEYLYSMETGEYYFLELNPRLQVEHPVTESIAEVNLPAAQVAVGMGIPLWQIPEIRRFYGMDNGGGYDIWRKTAALATPFNFDEVDSQWPKGHCVAVRITSENPDDGFKPTGGKVKEISFKSKPNVWGYFSVKSGGGIHEFADSQFGHVFAYGETRSAAITSMSLALKEIQIRGEIHTNVDYTVDLLNAPDFRENTIHTGWLDTRIAMRVQAERPPWYISVVGGALYKTITTNAETVSEYVSYLIKGQIPPKHISLVHSTISLNIEESKYTIEIVRSGQGSYRLRLNGSLIEANVQTLCDGGLLMQLDGNSHVIYAEEEAGGTRLLIDGKTCLLQNDHDPSRLLAETPCKLLRFLIADGAHVDADVPYAEVEVMKMCMPLLSPAAGVINVLLSEGQAMQAGDLIARLDLDDPSAVKRAEPFEGSFPEMSLPIAASGQVHKRCAASLNAARMVLAGYDHAANKVVQDLVWCLDTPALPFLQWEELMSVLATRLPRRLKSELEGKYNEYKLNVDHVKIKDFPTEMLRETIEENLACVSEKEMVTIERLVDPLMSLLKSYEGGRESHAHFIVKSLFEEYLSVEELFSDGIQSDVIERLRLQYSKDLQKVVDIVLSHQGVRNKTKLILALMEKLVYPNPAAYRDQLIRFSSLNHKRYYKLALKASELLEQTKLSELRTSIARNLSALDMFTEEKADFSLQDRKLAINESMGDLVTAPLPVEDALVSLFDCTDQTLQQRVIETYISRLYQPQLVKDSIQLKYQDSGVIALWEFTEGNHEKRLGAMVILKSLESVSTAIGAALKDASHYASSAGNTVHIALLDADTQLNTTEDSGDNDQAQDKMDKLSFVLKQDVVMADLRAADVKVVSCIVQRDGAIMPMRRTFLLSEEKLCYEEEPILRHVEPPLSALLELDKLKVKGYNEMKYTPSRDRQWHIYTLRNTENPKMLHRVFFRTLVRQPSAGNRFTSDHITDVEVGHAEEPLSFTSSSILKSLMIAKEELELHAIRTGHSHMYLCILKEQKLLDLVPVSGNTVVDVGQDEATACSLLKEMALKIHELVGARMHHLSVCQWEVKLKLVSDGPASGSWRVVTTNVTGHTCTVDIYREVEDTESQKLVYHSTALSSGPLHGVALNTSYQPLSVIDLKRCSARNNKTTYCYDFPLTFEAAVQKSWSNISSENNQCYVKATELVFAEKNGSWGTPIIPMQRAAGLNDIGMVAWILDMSTPEFPSGRQIIVIANDITFRAGSFGPREDAFFEAVTNLACEKKLPLIYLAANSGARIGIADEVKSCFRVGWTDDSSPERGFRYIYMTDEDHDRIGSSVIAHKMQLDSGEIRWVIDSVVGKEDGLGVENIHGSAAIASAYSRAYEETFTLTFVTGRTVGIGAYLARLGIRCIQRIDQPIILTGFSALNKLLGREVYSSHMQLGGPKIMATNGVVHLTVPDDLEGVSNILRWLSYVPANIGGPLPITKSLDPIDRPVAYIPENTCDPRAAISGIDDSQGKWLGGMFDKDSFVETFEGWAKTVVTGRAKLGGIPVGVIAVETQTMMQLVPADPGQPDSHERSVPRAGQVWFPDSATKTAQAMLDFNREGLPLFILANWRGFSGGQRDLFEGNLQAGSTIVENLRTYNQPAFVYIPKAAELRGGAWVVIDSKINPDRIECYAERTAKGNVLEPQGLIEIKFRSEELKECMGRLDPELIDLKARLQGANGSLSDGESLQKSIEARKKQLLPLYTQIAVRFAELHDTSLRMAAKGVIRKVVDWEDSRSFFYKRLRRRLSEDVLAKEIRGVIGEKFPHKSAIELIKKWYLASEAAAAGSTDWDDDDAFVAWRENPENYKEYIKELRAQRVSRLLSDVAGSSSDLQALPQGLSMLLDKMDPSKRAQFIEEVMKVLK

SEQ ID NO: 15 - DNA, 12683 bp, Alopecurus myosuroides Huds
tcagtttatggcagtctgtgtttgaagaacactgcaactccgctgtctgtccaaagggaggacgatgggatccacacatctgcccattgtcgggtttaatgcatccacaacaccatcgctatccactcttcgccagataaactcagctgctgctgcattccaatcttcgtccccttcaaggtcatccaagaagaaaagccgacgtgttaagtcaataagggatgatggcgatggaagcgtgccagaccctgcaggccatggccagtctattcgccaaggtgaacctaggaccatctccttacttttttgtcgtcaacctcagacttgcatagatttactttcttgattgagagcatgcttgttttagtgtaagatatctcaatactgtatcacaaaatgatagttaagaacaaatcactacaccaatcttcacatattgttcttattgggtttgctaaatcttagttcgcattagatttttttatgtctatgtcgacaccctgagcctccccgtgtctctgcattgagattcaagcagggattagggaaatcacgactggatcagaaggcaagcaccatcgccttagccataattaaatctctgtcaacctaggtgtagatggactctgtttttaatattcagtatgatgttttcttaagggagagggacacaaaaatatagtaagtagaagccttaccttcggaaaatacccatttaacctctgggagcatttgctactgcctagaaaaatccactttttaaagtttcaataattgcaaagacaagttactatgtgatagtacaaagtttggtggagaaacaactttttggtctatgtaataaaaaagacaaatatatgacacatgtatgttgcagtttaagaatttatgactgaatgttttgatgatataatagttctggaaaagaaggatgcctagattttgttttttgataaatgtagttataaaattcgaaaggttggcaaaccattgcttcttcttagctattgtgttggcttgctcagtttccaatgcatatctggatgtaggtctcgctggcatcatcgacctcccaaaggagggcgcatcagctccagatgtggacatttcacagtaagtacctcagcacactcacattatagcttagttctcttgaaagaacagcaaaaatgtataacgcatgtatagttcctagatttcacttgtcttattatcgttacgctgaaatgttgaagttgtaaattcgttattctcatagatttacacctctatgtacatctatgcactatgcacctgctgtgagttctggaaattgaaccattcagcgcactgcaatctgtaaggttttgtttttatataatatggttataaatcatgttcaacctctgcatctacaacattatttatgtgtggtatagtatatagtaatgttacagggtgagattttgctatataagttatgaaacttgtgttcaactttgtaaagggaaacatcctcaaacctgttcttagtggttacagcccaggcacatggccgttgcactgtatggagtattgttgggcacttacaaaacattttattggaaagattttttgatataagtattgtttaaatttaattgccaactgaaacccttacccggataacaagatgaataacccacttgcgtttttgattcatactaggcattactacgtcatatgtattacggtgaccgcagtaataactttgctctttcttttctagtgggtctgaagaccacaaggcctcctaccaaatgaatgggatactgaatgaatcacataacgggaggcacgcctctctgtctaaagtttatgaattttgcacggaattgggtggaaaaacaccaattcacagtgtattagtcgccaacaatggaatggcagcagctaagttcatgcggagtgtccggacatgggctaatgatacatttgggtcagagaaggcgattcagttgatagctatggcaactccggaagacatgagaataaatgcagagcacattagaattgctgatcagtttgttgaagtacctggtggaacaaacaataacaactatgcaaatgtccaactcatagtggaggtcagtactggtcatcccttgatgtgcagttatgcacaagctcctctttggtctttagcatgacatggcaacttcacttttgcagatagcagagagaactggtgtctccgccgtttggcctggttggggccatgcatctgagaatcctgaacttccagatgcactaactgcaaaaggaattgtttttcttgggccaccagcatcatcaatgaacgcactaggcgacaaggttggttcagctctcattgctcaagcagcaggggttcccactcttgcttggagtggatcacacgtaagcctcacattctctctgataaatcatcacctgatatttgtggtggatgcattatgtaacctatgacatttttattataggtggaaattccattagaactttgtttggactcgatacctgaggagatgtataggaaagcctgtgttacaaccgctgatgaagcagttgcaagttgtcagatgattggttaccctgccatgatcaaggcatcctggggtggtggtggtaaagggattagaaaggtacattattcatttgattggactgtacacaagagattgtgtgggctgtgatattttgtgcacagtgttagccctaacctttttaacatattaactcgatatctcttgcaggttaataatgatgacgaggtgaaagcactgtttaagcaagtacagggtgaagttcctggctccccgatatttatcatgagacttgcatctcaggttagacttctctagaagttctattttccaagcgtgctgtatctgggttgtatattgtacgtatggaagctttatttgctctttcttacaggctaaaattgtatcctgtaatctgtactaatattgtaattttcatttaaatccctctcccctttccctttgtagagtcgtcatcttgaagtccagctgctttgtgatgaatatggcaatgtagcagcacttcacagtcgtgattgcagtgtgcaacgacgacaccaaaaggtatgctgctccaaactgaaatcatcacttttatttcggttctgctttacgtgtagttttgatcaaatggttcaactgtgtccattttgtttgtttataacagattatcgaggaaggaccagttactgttgctcctcgtgaaacagtgaaagagctagagcaagcagcaaggaggcttgctaaggccgtgggttacgtcggtgctgctactgttgaatatctctacagcatggagactggtgaatactattttctggagcttaatccacggttgcaggtttgttcttttggacactctccaggacttctattttgttggcagtcgtttacattgttaaatggtctatattcaggttgagcacccagtcaccgagtcgatagctgaagtaaatttgcctgcagcccaagttgcagttgggatgggtatacccctttggcagattccaggtaataataatatcattgtaaagagtttcgtttctgtcccatgttctttctgtctaactatctccttattcagagatcagacgtttctacggaatggacaatggaggaggctatgatatttggaggaaaacagcagctctcgctactccattcaactttgatgaagtagattctcaatggccgaagggtcattgtgtggcagttaggataaccagtgagaatccagatgatggattcaagcctactggtggaaaagtaaaggtgggatttcctaatgttatatctatgtttcaattacactacggttagtaaactgatctgatcttgatttttttcgtatatttcaggagataagttttaaaagtaagccaaatgtctggggatatttctcagttaaggtaagctgttcatagctctgttgcagggtcatcttgttttgagttccgcagaagattagtctgcaagatttttattcgaattagtattctcattttggtttttgactaagtattgatccaatcaacaaatattgtctctcccttcatctgttttcagtctggtggaggcattcatgaatttgcggattctcagtttggtatgtaaaatgtgacgtaatgaatattcctctttgctattcgtattgatccttacattggaattgctcctttcattacaggacatgtttttgcctatggagagactagatcagcagcaataaccagcatgtctcttgcactaaaagagattcaaattcgtggagaaattcatacaaacgttgattacacggttgatctcttgaatgtaagtaacaataacaatttgttgaatcctacttttgatgtgatacaaccattttacatccggttttccttcaaaataatcccattctgtggtttctcgtatctttaattcaggccccagacttcagagaaaacacgatccataccggttggctggataccagaatagctatgcgtgttcaagctgagaggcctccctggtatatttcagtggttggaggagctctatatgtaagatatgaaactatgttaatgttactgcaacttttggcaagccaatcttgaaaaacagtagtgtttaattgaaataattgttttgtgctgtagaaaacaataaccaccaatgcggagaccgtttctgaatatgttagctatctcatcaagggtcagattccaccaaaggtagtgtcttaatgggcttaaactctgtatattgcttgaaggtggacattgctgaccattgtttttgtgcagcatatatcccttgtccattcaactatttctttgaatatagaggaaagcaaatatacagtaagtgtgacattccttaaaaaaagactctcagttacaatgaaatgatacttacactgatgctcatctacaccatgccacagattgagattgtgaggagtggacagggtagctacagattgagaatgaatggatcacttattgaagccaatgtacaaacattatgtgatggaggccttttaatgcaggtaccttctttcttttacttgctcataaatgtgatataatgtctgctgaaagagttctgattctttagttgtaatgtctccagctggatggaaatagccatgttatttatgctgaagaagaagcgggtggtacacagcttcttattgatggaaaaacatgcttgctacaggtaagaatattctgtttgtttgctcctttataatcttagtgtttgatggtaggactttatattcttatttgtgactttttactgcattcacctcttgaccattagcacttcattttttacacttcatctgtattgcttctgctgtttctcaattatagttattccaatgaccactctttagtaattttaacaattgccaatttatcataatacggggcaaaaaagtaggtgtccttaacaccatgtcatgtaacctataataagcttgtgataaaatcatttgtgatataatagaacaattgaatactttatgatttctttcttacatgaatactttatgattcttgatgacgctgcactgtatcctaaactacataaattacaaatcgttttgcagaatgaccatgatccgtcaaggttattagctgagacaccctgcaaacttcttcgtttcttgattgccgatggtgctcatgttgatgctgatgtaccatacgcggaagttgaggttatgaagatgtgcatgcccctcttgtcgcctgctgctggtgtcattaatgttttgttgtctgagggccaggcgatgcaggttatattactgcccttttgttgcttctgctgataaaagccattgcatgtgaagcatctgaacttaatatattttgtttcaggctggtgatcttatagcgagacttgatctcgatgacccttctgctgtgaagagagctgagccatttgaaggatcttttccagaaatgagccttcctattgctgcttctggccaagttcacaaaagatgtgctgcaagtttgaacgctgctcgaatggtccttgcaggatatgaccatgcggccaacaaagtaaacatcaagacattttatctcatgtttcctgcttttctcaaataccattctttaatagtatgaattctggattattctgacttattggcattttctgccttttgctaccaaatggtttctaatctatagaagttcttgagcttgtctttgcaaatctcgatttaatgcttttcttgtatgttcatcatactcatttatgataggttgcatttatccttctgctattttcctttctctcagtaaatcatgatggatgctctttctgttatgttcatcatgctgtctattatccttgtgctatttttctatttccagtagtggatgtattggtttaataattcctgatcaaactttgtattttgttgttatttatacttggcttccttttcaggttgtgcaagatttggtatggtgccttgatacacctgctcttcctttcctacaatgggaagagcttatgtctgttttagcaactagacttccaagacgtcttaagagcgaggtatgtgataattgatatgatatgcagaatcaggcataaagggacattgatacatttaatttatgatatagaagggtcttcatcctcgattaaaagatcaattcacttatcatgatttacattctacattgttgaatcaccttggtaatttgccgtaacttattgggcaactattagcttttctaataacgtaatcaaaattcagaatattttacttcaattcttcgtaacatggaacatttggtacttcgtctcatttatttgcactgtacgctgttttagttggtttgccattctaactgaatctttaaagttcttacttatttggttttaacccagatcttgtttatttatcttttataactttcttatgttctgcctcaacggttcatactttttatgcatccagttggagggcaaatacaatgaatacaagttaaatgttgaccatgtgaagatcaaggatttccctaccgagatgcttagagagacaatcgaggtcagtttttgtttcttatggcatcccagtctaaattatactattttttgtaacaagttttcttttaggaaaatcttgcatgtgtttccgagaaggaaatggtgacaattgagaggcttgttgaccctctgatgaacctgctgaagtcatacgagggtgggagagaaagccatgcccactttattgtcaagtccctttttgaggagtatctctcggttgaggaactattcagtgatggcattcaggttatctaacacttctaaactgagcagatctactagagtcattttctaagggtcataattttccagaacctcttgggtgattaagtagcaaaaataatttgtacacgacttacgacttacttccttcgaaacacttttcactcattattttcctcaaaatgtgccattttgtagtctgacgtgattgaacgcctgcgcctacaatatagtaaagacctccagaaggttgtagacattgttttgtctcaccaggtaaactactttttggcctaatgacttggtgcaagtgatcacagaaacaatctttgttactgatagtttgatttgttctagggtgtgagaaacaaaacaaagctgatactcgcgctcatggagaaactggtctatccaaaccctgctgcctacagagatcagttgattcgcttttcttccctcaaccataaaagatattataaggtgacaatggcgacctaaagtaatggaagctttttgattaatttgttgtgatattttaggctaatgaattactttcattgtaattctgcagttggctcttaaagctagtgaacttcttgaacaaaccaagctcagcgaactccgcacaagcattgcaaggaacctttcaacgctggatatgttcaccgaggaaaaggcagatttctccttgcaagacagaaaattggccattaatgagagcatgggagatttagtcactgccccactgccagttgaagatgcacttgtttctttgtttgattgtactgatcaaactcttcagcagagagtgattgagacatacatatctcgattataccaggtattacatgagctatttttttctggattttattatactctctctcagcatttctggaagcataaactaaggttcctaatgaaataagatactcagtgtttcattaagataaatcctagataatctaggcgtgggaagatttgatttagaacttgtaggcatgttactgctctgtaagttggctaacttgccaatgatattttcagcctcaacttgtgaaggatagcatccagctgaaatatcaggattctggtgttattgctttatgggaattcactgaaggaaatcatgagaagagattgggtgctatggttatcctgaagtcactagaatctgtgtcaacagccattggagctgctctaaaggatgcatcacattatgcaagctctgcgggcaacacggtgcatattgctttgttggatgctgatacccaactgaatacaactgaagataggtatgttcatgtgcagtattagtgcagatgagtttatttggtgcaaaaataagttaatctatttctttcagtggtgataatgaccaagctcaagacaagatggataaactttcttttgtactgaaacaagatgttgtcatggctgatctacgtgctgctgatgtcaaggttgttagttgcattgttcaaagagatggagcaatcatgcctatgcgccgtaccttcctcttgtcagaggaaaaactttgttacgaggaagagccgattcttcggcatgtggagcctccactttctgcacttcttgagttggtatgcaactccatcaaactgactacgtgctgttttgatatattttaatgctttcactttgttatttgctacttgtattcacttagcttgctgtggatacaggataaattgaaagtgaaaggatacaatgagatgaagtatacaccgtcacgtgatcgtcagtggcatatatacacacttagaaatactgaaaatccaaaaatgctgcacagggtatttttccgaacactagtcagacaacccagtgcaggcaacaggtttacatcagaccatatcactgatgttgaagtaggacacgcagaggaacctctttcatttacttcaagcagcatattaaaatcgttgatgattgctaaagaagaattggagcttcacgcgatcaggactggccattctcatatgtacttgtgcatattgaaagagcaaaagcttcttgaccttgttcctgtttcagggtaagcctgcacatcgttctttttgcagaacatgtattccttgctcttgtgttttgccttctcaatgagcttttcatcgtactcaggaacactgttgtggatgttggtcaagatgaagctactgcatgctctcttttgaaagaaatggctttaaagatacatgaacttgttggtgcaagaatgcatcatctttctgtttgccagtgggaagtgaaacttaagttggtgagcgatgggcctgccagtggtagctggagagttgtaacaaccaatgttactggtcacacctgcactgtggatgtgagttttatctccttgcttcctgtttttctgcatggaactaatgaaactgaagtgaacatattatatatgtgacatacatatgactatcatctttgattatcataaaaaaagaactatcatcttcgtttagtttgttgtcatttccacctcatttttggtctgaatctcatggtgcttttaatgcttttagatctaccgggaggtcgaagatacagaatcacagaaactagtataccactccaccgcattgtcatctggtcctttgcatggtgttgcactgaatacttcgtatcagcctttgagtgttattgatttaaaacgttgctctgccaggaacaacaaaactacatactgctatgattttccattggttagtatctatctctctctatatgtattatgttagcaggttcttattggtattacatgtcctaaatctgacaacaactcaaaatgtagacatttgaagctgcagtgcagaagtcgtggtctaacatttccagtgaaaacaaccaatgttatgttaaagcgacagagcttgtgtttgctgaaaagaatgggtcgtggggcactcctataattcctatgcagcgtgctgctgggctgaatgacattggtatggtagcctggatcttggacatgtccactcctgaatttcccagcggcagacagatcattgttatcgcaaatgatattacatttagagctggatcatttggcccaagggaagatgcatttttcgaagctgtaaccaacctggcttgtgagaagaagcttccacttatctacttggctgcaaactctggtgctcggattggcattgctgatgaagtaaaatcttgcttccgtgttggatggactgatgatagcagccctgaacgtggatttaggtacatttatatgactgacgaagaccatgatcgtataggctcttcagttatagcacacaagatgcagctagatagtggcgagatcaggtgggttatcgattctgttgtgggaaaagaggatggactaggtgtggagaacatacatggaagtgctgctattgccagtgcctattctagggcgtacgaggagacatttacacttacattcgttactggacgaactgttggaatcggagcctatcttgctcgacttggcatacggtgcatacagcgtattgaccagcccattattttgaccgggttttctgccctgaacaagcttcttgggcgggaggtgtacagctcccacatgcagttgggtggtcccaaaatcatggcgacgaatggtgttgtccatctgactgttccagatgaccttgaaggtgtttctaatatattgaggtggctcagctatgttcctgcaaacattggtggacctcttcctattacaaaatctttggacccaatagacagacccgttgcatacatccctgagaatacatgtgatcctcgtgcagccatcagtggcattgatgacagccaagggaaatggttgggtggcatgtttgacaaagacagttttgtggagacatttgaaggatgggcgaagacagtagttactggcagagcaaaacttggagggattcctgttggtgttatagctgtggagacacagaccatgatgcagctcgtccccgctgatccaggccagcctgattcccatgagcggtctgttcctcgtgctgggcaagtttggtttccagattctgctaccaagacagcgcaggcgatgttggacttcaaccgtgaaggattacctctgttcatacttgctaactggagaggcttctctggagggcaaagagatctttttgaaggaaatctgcaggctgggtcaacaattgttgagaaccttaggacatacaatcagcctgcctttgtatatatccccaaggctgcagagctacgtggaggagcctgggtcgtgattgatagcaagataaacccagatcgcatcgagtgctatgctgagaggactgcaaagggtaatgttctcgaacctcaagggttgattgagatcaagttcaggtcagaggaactcaaagaatgcatgggtaggcttgatccagaattgatagatctgaaagcaagactccagggagcaaatggaagcctatctgatggagaatcccttcagaagagcatagaagctcggaagaaacagttgctgcctctgtacacccaaatcgcggtacgttttgcggaattgcacgacacttcccttagaatggctgctaaaggtgtgatcaggaaagttgtagactgggaagactctcggtctttcttctacaagagattacggaggaggctatccgaggacgttctggcaaaggagattagaggtgtaattggtgagaagtttcctcacaaatcagcgatcgagctgatcaagaaatggtacttggcttccgaggcagctgcagcaggaagcaccgactgggatgacgacgatgcttttgtcgcctggagggagaaccctgaaaactataaggagtatatcaaagagcttagggctcaaagggtatctcggttgctctcagatgttgcaggctccagttcggatttacaagccttgccgcagggtctttccatgctactagataaggtacgcatacttacagttttacctgcatctgtttatttgcaagtattttatcgaggttgagtaaaatgctgctatcttcatatacacttgtatgtcctgctatcttattcaaatatagtatcttaccaaataatatctaagacgctggatactttgttcagatggatccctctaagagagcacagtttatcgaggaggtcatgaaggtcctgaaatgatcaaatgataccaacacatccaatacagtatgtgcatgatatctgtttctcttgaagtacatatatagatggatacaaggcggctgtaactgatggtagctaatctgggccaaccattacttttgtgaacttgctggtggtctttattattcaaggcacagctcgccttcggaccccctc

SEQ ID NO: 16 - protein, 2320 aa, Alopecurus myosuroides Huds
MGSTHLPIVGFNASTTPSLSTLRQINSAAAAFQSSSPSRSSKKKSRRVKSIRDDGDGSVPDPAGHGQSIRQGLAGIIDLPKEGASAPDVDISHGSEDHKASYQMNGILNESHNGRHASLSKVYEFCTELGGKTPIHSVLVANNGMAAAKFMRSVRTWANDTFGSEKAIQLIAMATPEDMRINAEHIRIADQFVEVPGGTNNNNYANVQLIVEIAERTGVSAVWPGWGHASENPELPDALTAKGIVFLGPPASSMNALGDKVGSALIAQAAGVPTLAWSGSHVEIPLELCLDSIPEEMYRKACVTTADEAVASCQMIGYPAMIKASWGGGGKGIRKVNNDDEVKALFKQVQGEVPGSPIFIMRLASQSRHLEVQLLCDEYGNVAALHSRDCSVQRRHQKIIEEGPVTVAPRETVKELEQAARRLAKAVGYVGAATVEYLYSMETGEYYFLELNPRLQVEHPVTESIAEVNLPAAQVAVGMGIPLWQIPEIRRFYGMDNGGGYDIWRKTAALATPFNFDEVDSQWPKGHCVAVRITSENPDDGFKPTGGKVKEISFKSKPNVWGYFSVKSGGGIHEFADSQFGHVFAYGETRSAAITSMSLALKEIQIRGEIHTNVDYTVDLLNAPDFRENTIHTGWLDTRIAMRVQAERPPWYISVVGGALYKTITTNAETVSEYVSYLIKGQIPPKHISLVHSTISLNIEESKYTIEIVRSGQGSYRLRMNGSLIEANVQTLCDGGLLMQLDGNSHVIYAEEEAGGTQLLIDGKTCLLQNDHDPSRLLAETPCKLLRFLIADGAHVDADVPYAEVEVMKMCMPLLSPAAGVINVLLSEGQAMQAGDLIARLDLDDPSAVKRAEPFEGSFPEMSLPIAASGQVHKRCAASLNAARMVLAGYDHAANKVVQDLVWCLDTPALPFLQWEELMSVLATRLPRRLKSELEGKYNEYKLNVDHVKIKDFPTEMLRETIEENLACVSEKEMVTIERLVDPLMNLLKSYEGGRESHAHFIVKSLFEEYLSVEELFSDGIQSDVIERLRLQYSKDLQKVVDIVLSHQGVRNKTKLILALMEKLVYPNPAAYRDQLIRFSSLNHKRYYKLALKASELLEQTKLSELRTSIARNLSTLDMFTEEKADFSLQDRKLAINESMGDLVTAPLPVEDALVSLFDCTDQTLQQRVIETYISRLYQPQLVKDSIQLKYQDSGVIALWEFTEGNHEKRLGAMVILKSLESVSTAIGAALKDASHYASSAGNTVHIALLDADTQLNTTEDSGDNDQAQDKMDKLSFVLKQDVVMADLRAADVKVVSCIVQRDGAIMPMRRTFLLSEEKLCYEEEPILRHVEPPLSALLELDKLKVKGYNEMKYTPSRDRQWHIYTLRNTENPKMLHRVFFRTLVRQPSAGNRFTSDHITDVEVGHAEEPLSFTSSSILKSLMIAKEELELHAIRTGHSHMYLCILKEQKLLDLVPVSGNTVVDVGQDEATACSLLKEMALKIHELVGARMHHLSVCQWEVKLKLVSDGPASGSWRVVTTNVTGHTCTVDIYREVEDTESQKLVYHSTALSSGPLHGVALNTSYQPLSVIDLKRCSARNNKTTYCYDFPLTFEAAVQKSWSNISSENNQCYVKATELVFAEKNGSWGTPIIPMQRAAGLNDIGMVAWILDMSTPEFPSGRQIIVIANDITFRAGSFGPREDAFFEAVTNLACEKKLPLIYLAANSGARIGIADEVKSCFRVGWTDDSSPERGFRYIYMTDEDHDRIGSSVIAHKMQLDSGEIRWVIDSVVGKEDGLGVENIHGSAAIASAYSRAYEETFTLTFVTGRTVGIGAYLARLGIRCIQRIDQPIILTGFSALNKLLGREVYSSHMQLGGPKIMATNGVVHLTVPDDLEGVSNILRWLSYVPANIGGPLPITKSLDPIDRPVAYIPENTCDPRAAISGIDDSQGKWLGGMFDKDSFVETFEGWAKTVVTGRAKLGGIPVGVIAVETQTMMQLVPADPGQPDSHERSVPRAGQVWFPDSATKTAQAMLDFNREGLPLFILANWRGFSGGQRDLFEGNLQAGSTIVENLRTYNQPAFVYIPKAAELRGGAWVVIDSKINPDRIECYAERTAKGNVLEPQGLIEIKFRSEELKECMGRLDPELIDLKARLQGANGSLSDGESLQKSIEARKKQLLPLYTQIAVRFAELHDTSLRMAAKGVIRKVVDWEDSRSFFYKRLRRRLSEDVLAKEIRGVIGEKFPHKSAIELIKKWYLASEAAAAGSTDWDDDDAFVAWRENPENYKEYIKELRAQRVSRLLSDVAGSSSDLQALPQGLSMLLDKMDPSKRAQFIEEVMKVLK